European Patent Specification EP 3 559 262 B1, published April 9, 2025. Title: ARRAYS WITH QUALITY CONTROL TRACERS. Applicant: Illumina, Inc. The sequence listing filed with the application follows.

SEQUENCE LISTING (26 sequences)

SEQ ID NO: 1 - DNA, 29 bp, Artificial Sequence
  primer_bind
aatgatacggcgaccaccgagauctacac

SEQ ID NO: 2 - DNA, 24 bp, Artificial Sequence
  primer_bind
  misc_feature (22)..(22): 8-oxo-guanine
caagcagaagacggcatacganat

SEQ ID NO: 3 - DNA, 29 bp, Artificial Sequence
  synthesized
catctaggcatctaagcatcaaucttaca

SEQ ID NO: 4 - DNA, 27 bp, Artificial Sequence
  synthesized
acatacatacatacatacauacataca

SEQ ID NO: 5 - DNA, 26 bp, Artificial Sequence
  synthesized
attgattgattgattgatugattgat

SEQ ID NO: 6 - DNA, 30 bp, Artificial Sequence
  misc_feature
  misc_feature (1)..(1): poly Thymine with a number of T bases ranging from 2-20
ncatctaggcatctaagcatcaaucttaca

SEQ ID NO: 7 - DNA, 28 bp, Artificial Sequence
  misc_feature
  misc_feature (1)..(1): poly Thymine with a number of T bases ranging from 2-20
nacatacatacatacatacauacataca

SEQ ID NO: 8 - DNA, 27 bp, Artificial Sequence
  misc_feature
  misc_feature (1)..(1): poly Thymine with a number of T bases ranging from 2-20
nattgattgattgattgatugattgat

SEQ ID NO: 9 - DNA, 30 bp, Artificial Sequence
  misc_feature
  misc_feature (30)..(30): red fluorescent dye attached to Adenine through Amino-modifier C6 dT linker
catctaggcatctaagcatcaaucttacan

SEQ ID NO: 10 - DNA, 28 bp, Artificial Sequence
  misc_feature
  misc_feature (28)..(28): red fluorescent dye attached to Adenine through Amino-modifier C6 dT linker
acatacatacatacatacauacatacan

SEQ ID NO: 11 - DNA, 27 bp, Artificial Sequence
  misc-Feature
  misc_feature (27)..(27): red fluorescent dye attached to Thymine through Amino-modifier C6 dT linker
attgattgattgattgatugattgatn

SEQ ID NO: 12 - DNA, 30 bp, Artificial Sequence; identical to SEQ ID NO: 9
  misc_feature
  misc_feature (30)..(30): xanthene fluorophore attached to Adenine through Amino-modifier C6 dT linker

SEQ ID NO: 13 - DNA, 28 bp, Artificial Sequence
  misc_feature
  misc_feature (28)..(28): xanthene fluorophore attached to Adenine through Amino-modifier C6 dT linker
acatacatacatacatacauacatacan

SEQ ID NO: 14 - DNA, 27 bp, Artificial Sequence
  misc_feature
  misc_feature (27)..(27): xanthene fluorophore attached to Thymine through Amino-modifier C6 dT linker
attgattgattgattgatugattgatn

SEQ ID NO: 15 - DNA, 34 bp, Artificial Sequence
  misc_feature
  misc_feature (34)..(34): xanthene fluorophore attached to Adenine through Amino-modifier C6 dT linker
ttttttacatacatacatacatacauacatacan

SEQ ID NO: 16 - DNA, 28 bp, Artificial Sequence
  synthesized
aatgatacggcgaccaccgagauctaca

SEQ ID NO: 17 - DNA, 28 bp, Artificial Sequence
  synthesized
aatgatacggcgaccaccgagaucacac

SEQ ID NO: 18 - DNA, 34 bp, Artificial Sequence
  synthesized
ttttttaatgatacggcgaccaccgagauctaca

SEQ ID NO: 19 - DNA, 34 bp, Artificial Sequence
  synthesized
ttttttaatgatacggcgaccaccgagaucacac

SEQ ID NO: 20 - DNA, 35 bp, Artificial Sequence
  sythesized
ttttttaatgatacggcgaccaccgagauctacac

SEQ ID NO: 21 - DNA, 35 bp, Artificial Sequence
  misc_feature
  misc_feature (35)..(35): xanthene fluorophore attached to adenine through Amino-modifier C6 dT linker
ttttttaatgatacggcgaccaccgagauctacan

SEQ ID NO: 22 - DNA, 30 bp, Artificial Sequence
  misc_feature
  misc_feature (30)..(30): xanthene fluorophore attached to Cytosine through Amino-modifier C6 dT linker
ttttttaatgatacggcgaccaccgagauc

SEQ ID NO: 23 - DNA, 36 bp, Artificial Sequence
  misc_feature
  misc_feature (36)..(36): xanthene fluorophore attached to Cytosine through Amino-modifier C6 dT linker
ttttttaatgatacggcgaccaccgagauctacacn

SEQ ID NO: 24 - DNA, 29 bp, Artificial Sequence
  misc_feature
  misc_feature (29)..(29): red fluorescent dye attached to adenine through Amino-modifier C6 dT linker
aatgatacggcgaccaccgagauctacan

SEQ ID NO: 25 - DNA, 31 bp, Artificial Sequence
  misc_feature
  misc_feature (1)..(1): poly Thymine with a number of T bases ranging from 2-20
  misc_feature (31)..(31): red fluorescent dye attached to adenine through Amino-modifier C6 dT linker
ncatctaggcatctaagcatcaaucttacan

SEQ ID NO: 26 - DNA, 30 bp, Artificial Sequence
  misc_feature
  misc_feature (1)..(1): poly Thymine with a number of T bases ranging from 2-20
  misc_feature (30)..(30): red fluorescent dye attached to adenine through Amino-modifier C6 dT linker
naatgatacggcgaccaccgagauctacan